European Patent Application EP 4 545 969 A2, published April 30, 2025. Title: PEPTIDE WITH NEUTRALIZING ACTIVITY AGAINST SEVERE ACUTE RESPIRATORY SYNDROME CORONAVIRUS 2. Applicant: CAREGEN CO., LTD. The sequence listing filed with the application follows.

SEQUENCE LISTING (6 sequences)

SEQ ID NO: 1 - protein, 11 aa, synthetic construct
RSYMTTHHEQF

SEQ ID NO: 2 - protein, 7 aa, synthetic construct
KFNRRHH

SEQ ID NO: 3 - protein, 12 aa, synthetic construct
KYLLVHRPYYRR

SEQ ID NO: 4 - protein, 12 aa, synthetic construct
WVPYQARVPYPR

SEQ ID NO: 5 - protein, 12 aa, synthetic construct
RLYCKNGGFFLR

SEQ ID NO: 6 - protein, 9 aa, synthetic construct
KHRGGGNRR